European Patent Application EP 4 488 285 A2, published January 8, 2025. Title: MOLECULAR HOPPER. Applicant: Oxford University Innovation Limited. The sequence listing filed with the application follows.

SEQUENCE LISTING (19 sequences)

SEQ ID NO: 1 - protein, 293 aa, Staphylococcus aureus
ADSDINIKTGTTDIGSNTTVKTGDLVTYDKENGMHKKVFYSFIDDKNHNKKLLVIRTKGTIAGQYRVYSEEGANKSGLAWPSAFKVQLQLPDNEVAQISDYYPRNSIDTKEYMSTLTYGFNGNVTGDDTGKIGGLIGANVSIGHTLKYVQPDFKTILESPTDKKVGWKVIFNNMVNQNWGPYDRDSWNPVYGNQLFMKTRNGSMKAADNFLDPNKASSLLSSGFSPDFATVITMDRKASKQQTNIDVIYERVRDDYQLHWTSTNWKGTNTKDKWTDRSSERYKIDWEKEEMTN

SEQ ID NO: 2 - protein, 307 aa, synthetic construct
  REGION 1..307: note = alpha hemolysin mutant (WT-D8H6)
ADSDINIKTGTTDIGSNTTVKTGDLVTYDKENGMHKKVFYSFIDDKNHNKKLLVIRTKGTIAGQYRVYSEEGANKSGLAWPSAFKVQLQLPDNEVAQISDYYPRNSIDTKEYMSTLTYGFNGNVTGDDTGKIGGLIGANVSIGHTLKYVQPDFKTILESPTDKKVGWKVIFNNMVNQNWGPYDRDSWNPVYGNQLFMKTRNGSMKAADNFLDPNKASSLLSSGFSPDFATVITMDRKASKQQTNIDVIYERVRDDYQLHWTSTNWKGTNTKDKWTDRSSERYKIDWEKEEMTNDDDDDDDDHHHHHH

SEQ ID NO: 3 - protein, 307 aa, synthetic construct
  REGION 1..307: note = alpha hemolysin mutant (115C117C-D8H6)
ADSDINIKTGTTDIGSNTTVKTGDLVTYDKENGMHKKVFYSFIDDKNHNKKLLVIRTKGTIAGQYRVYSEEGANKSGLAWPSAFKVQLQLPDNEVAQISDYYPRNSIDTKEYMSCLCYGFNGNVTGDDTGKIGGLIGANVSIGHTLKYVQPDFKTILESPTDKKVGWKVIFNNMVNQNWGPYDRDSWNPVYGNQLFMKTRNGSMKAADNFLDPNKASSLLSSGFSPDFATVITMDRKASKQQTNIDVIYERVRDDYQLHWTSTNWKGTNTKDKWTDRSSERYKIDWEKEEMTNDDDDDDDDHHHHHH

SEQ ID NO: 4 - protein, 307 aa, synthetic construct
  REGION 1..307: note = alpha hemolysin mutant (115C117C119C-D8H6)
ADSDINIKTGTTDIGSNTTVKTGDLVTYDKENGMHKKVFYSFIDDKNHNKKLLVIRTKGTIAGQYRVYSEEGANKSGLAWPSAFKVQLQLPDNEVAQISDYYPRNSIDTKEYMSCLCYCFNGNVTGDDTGKIGGLIGANVSIGHTLKYVQPDFKTILESPTDKKVGWKVIFNNMVNQNWGPYDRDSWNPVYGNQLFMKTRNGSMKAADNFLDPNKASSLLSSGFSPDFATVITMDRKASKQQTNIDVIYERVRDDYQLHWTSTNWKGTNTKDKWTDRSSERYKIDWEKEEMTNDDDDDDDDHHHHHH

SEQ ID NO: 5 - protein, 307 aa, synthetic construct
  REGION 1..307: note = alpha hemolysin mutant (113C115C117C119C121C-D8H6)
ADSDINIKTGTTDIGSNTTVKTGDLVTYDKENGMHKKVFYSFIDDKNHNKKLLVIRTKGTIAGQYRVYSEEGANKSGLAWPSAFKVQLQLPDNEVAQISDYYPRNSIDTKEYCSCLCYCFCGNVTGDDTGKIGGLIGANVSIGHTLKYVQPDFKTILESPTDKKVGWKVIFNNMVNQNWGPYDRDSWNPVYGNQLFMKTRNGSMKAADNFLDPNKASSLLSSGFSPDFATVITMDRKASKQQTNIDVIYERVRDDYQLHWTSTNWKGTNTKDKWTDRSSERYKIDWEKEEMTNDDDDDDDDHHHHHH

SEQ ID NO: 6 - protein, 307 aa, synthetic construct
  REGION 1..307: note = alpha hemolysin mutant (113C115C117C119C121C123C-D8H6)
ADSDINIKTGTTDIGSNTTVKTGDLVTYDKENGMHKKVFYSFIDDKNHNKKLLVIRTKGTIAGQYRVYSEEGANKSGLAWPSAFKVQLQLPDNEVAQISDYYPRNSIDTKEYCSCLCYCFCGCVTGDDTGKIGGLIGANVSIGHTLKYVQPDFKTILESPTDKKVGWKVIFNNMVNQNWGPYDRDSWNPVYGNQLFMKTRNGSMKAADNFLDPNKASSLLSSGFSPDFATVITMDRKASKQQTNIDVIYERVRDDYQLHWTSTNWKGTNTKDKWTDRSSERYKIDWEKEEMTNDDDDDDDDHHHHHH

SEQ ID NO: 7 - protein, 307 aa, synthetic construct
  REGION 1..307: note = alpha hemolysin mutant (115C117C119C139C-D8H6)
ADSDINIKTGTTDIGSNTTVKTGDLVTYDKENGMHKKVFYSFIDDKNHNKKLLVIRTKGTIAGQYRVYSEEGANKSGLAWPSAFKVQLQLPDNEVAQISDYYPRNSIDTKEYMSCLCYCFNGNVTGDDTGKIGGLIGACVSIGHTLKYVQPDFKTILESPTDKKVGWKVIFNNMVNQNWGPYDRDSWNPVYGNQLFMKTRNGSMKAADNFLDPNKASSLLSSGFSPDFATVITMDRKASKQQTNIDVIYERVRDDYQLHWTSTNWKGTNTKDKWTDRSSERYKIDWEKEEMTNDDDDDDDDHHHHHH

SEQ ID NO: 8 - DNA, 36 bp, synthetic construct
  misc_feature 1..36: note = forward mutagenic primer
  source 1..36: mol_type = other DNA
ctgcttctgcggttgtgttactggtgatgatacagg

SEQ ID NO: 9 - DNA, 23 bp, synthetic construct
  misc_feature 1..23: note = reverse non-mutagenic primer (SC47)
  source 1..23: mol_type = other DNA
cagaagtggtcctgcaactttat

SEQ ID NO: 10 - DNA, 36 bp, synthetic construct
  misc_feature 1..36: note = reverse mutagenic primer
  source 1..36: mol_type = other DNA
cctgtatcatcaccagtaacacaaccgcagaagcag

SEQ ID NO: 11 - DNA, 23 bp, synthetic construct
  misc_feature 1..23: note = forward non-mutagenic primer (SC46)
  source 1..23: mol_type = other DNA
ataaagttgcaggaccacttctg

SEQ ID NO: 12 - DNA, 39 bp, synthetic construct
  misc_feature 1..39: note = forward mutagenic primer
  source 1..39: mol_type = other DNA
caaaagagtatatgagttgcttatgctattgcttcaacg

SEQ ID NO: 13 - DNA, 39 bp, synthetic construct
  misc_feature 1..39: note = reverse mutagenic primer
  source 1..39: mol_type = other DNA
cgttgaagcaatagcataagcaactcatatactcttttg

SEQ ID NO: 14 - DNA, 37 bp, synthetic construct
  misc_feature 1..37: note = forward mutagenic primer
  source 1..37: mol_type = other DNA
ccttattggtgcatgtgtttcgattggtcatacactg

SEQ ID NO: 15 - DNA, 37 bp, synthetic construct
  misc_feature 1..37: note = reverse mutagenic primer
  source 1..37: mol_type = other DNA
cagtgtatgaccaatcgaaacacatgcaccaataagg

SEQ ID NO: 16 - DNA, 36 bp, synthetic construct
  source 1..36: mol_type = other DNA
  misc_feature 1..36: note = forward mutagenic primer
caaatgtttcgatttgtcatacactgaaatatgttc

SEQ ID NO: 17 - DNA, 36 bp, synthetic construct
  source 1..36: mol_type = other DNA
  misc_feature 1..36: note = reverse mutagenic primer
gaacatatttcagtgtatgacaaatcgaaacatttg

SEQ ID NO: 18 - DNA, 36 bp, synthetic construct
  source 1..36: mol_type = other DNA
  misc_feature 1..36: note = forward mutagenic primer
cggattcaacggttgtgttactggtgatgatacagg

SEQ ID NO: 19 - DNA, 36 bp, synthetic construct
  source 1..36: mol_type = other DNA
  misc_feature 1..36: note = reverse mutagenic primer
cctgtatcatcaccagtaacacaaccgttgaatccg